European Patent Application EP 4 445 952 A2, published October 16, 2024. Title: SUNITINIB FORMULATIONS AND METHODS FOR USE THEREOF IN TREATMENT OF GLAUCOMA. Applicant: The Johns Hopkins University. The sequence listing filed with the application follows.

SEQUENCE LISTING (2 sequences)

SEQ ID NO: 1 - DNA, 20 bp, synthetic construct
  misc_feature 1..20: note = Synthetic Primer
  source 1..20: mol_type = other DNA
attcctcagccatcatctgg

SEQ ID NO: 2 - DNA, 20 bp, synthetic construct
  misc_feature 1..20: note = Synthetic Primer
  source 1..20: mol_type = other DNA
atttcgtggtttgctgttcc